European Patent Specification EP 4 051 694 B1, published July 2, 2025. Title: AAV Vector Variants for Ocular Gene Delivery. Applicant: Universität Bern. The sequence listing filed with the application follows.

SEQUENCE LISTING (28 sequences)

SEQ ID NO: 1 - protein, 735 aa, Artificial Sequence
  AAV2 capsid protein VP1 with different mutations
MAADGYLPDWLEDTLSEGIRQWWKLKPGPPPPKPAERHKDDSRGLVLPGYKYLGPFNGLDKGEPVNEADAAALEHDKAYDRQLDSGDNPYLKYNHADAEFQERLKEDTSFGGNLGRAVFQAKKRVLEPLGLVEEPVKTAPGKKRPVEHSPVEPDSSSGTGKAGQQPARKRLNFGQTGDADSVPDPQPLGQPPAAPSGLGTNTMATGSGAPMADNNEGADGVGNSSGNWHCDSTWMGDRVITTSTRTWALPTFNNHLYKQISSQSGASNDNHFFGYSTPWGYFDFNRFHCHFSPRDWQRLINNNWGFRPKRLNFKLFNIQVKEVTQNDGTTTIANNLTSTVQVFTDSEYQLPYVLGSAHQGCLPPFPADVFMVPQYGYLTLNNGSQAVGRSSFYCLEYFPSQMLRTGNNFTFSYTFEDVPFHSSYAHSQSLDRLMNPLIDQYLYFLSRTNTPSGTTTQSRLQFSQAGASDIRDQSRNWLPGPCYRQQRVSKTSADNNNSEFSWTGATKYHLNGRDSLVNPGPAMASHKDDEEKFFPQSGVLIFGKQGSEKTNVDIEKVMITDEEEIRTTNPVATEQYGSVSTNLQRGNRQAATADVNTQGVLPGMVWQDRDVYLQGPIWAKIPHTDGHFHPSPLMGGFGLKHPPPQILIKNTPVPANPSTTFSAAKFASFITQYSTGQVSVEIEWELQKENSKRWNPEIQFTSNYNKSVNVDFTVDTNGVYSEPRPIGTRFLTRNL

SEQ ID NO: 2 - protein, 747 aa, Artificial Sequence
  AAV2 capsid protein VP1 with insertion
MAADGYLPDWLEDTLSEGIRQWWKLKPGPPPPKPAERHKDDSRGLVLPGYKYLGPFNGLDKGEPVNEADAAALEHDKAYDRQLDSGDNPYLKYNHADAEFQERLKEDTSFGGNLGRAVFQAKKRVLEPLGLVEEPVKTAPGKKRPVEHSPVEPDSSSGTGKAGQQPARKRLNFGQTGDADSVPDPQPLGQPPAAPSGLGTNTMATGSGAPMADNNEGADGVGNSSGNWHCDSTWMGDRVITTSTRTWALPTFNNHLYKQISSQSGASNDNHFFGYSTPWGYFDFNRFHCHFSPRDWQRLINNNWGFRPKRLNFKLFNIQVKEVTQNDGTTTIANNLTSTVQVFTDSEYQLPYVLGSAHQGCLPPFPADVFMVPQYGYLTLNNGSQAVGRSSFYCLEYFPSQMLRTGNNFTFSYTFEDVPFHSSYAHSQSLDRLMNPLIDQYLYFLSRTNTPSGTTTQSRLQFSQAGASDIRDQSRNWLPGPCYRQQRVSKTSADNNNSEFSWTGATKYHLNGRDSLVNPGPAMASHKDDEEKFFPQSGVLIFGKQGSEKTNVDIEKVMITDEEEIRTTNPVATEQYGSVSTNLQRGNAAASASEASTAARQAATADVNTQGVLPGMVWQDRDVYLQGPIWAKIPHTDGHFHPSPLMGGFGLKHPPPQILIKNTPVPANPSTTFSAAKFASFITQYSTGQVSVEIEWELQKENSKRWNPEIQFTSNYNKSVNVDFTVDTNGVYSEPRPIGTRFLTRNL

SEQ ID NO: 3 - protein, 747 aa, Artificial Sequence
  AAV2 capsid protein VP1 with insertion
MAADGYLPDWLEDTLSEGIRQWWKLKPGPPPPKPAERHKDDSRGLVLPGYKYLGPFNGLDKGEPVNEADAAALEHDKAYDRQLDSGDNPYLKYNHADAEFQERLKEDTSFGGNLGRAVFQAKKRVLEPLGLVEEPVKTAPGKKRPVEHSPVEPDSSSGTGKAGQQPARKRLNFGQTGDADSVPDPQPLGQPPAAPSGLGTNTMATGSGAPMADNNEGADGVGNSSGNWHCDSTWMGDRVITTSTRTWALPTFNNHLYKQISSQSGASNDNHFFGYSTPWGYFDFNRFHCHFSPRDWQRLINNNWGFRPKRLNFKLFNIQVKEVTQNDGTTTIANNLTSTVQVFTDSEYQLPYVLGSAHQGCLPPFPADVFMVPQYGYLTLNNGSQAVGRSSFYCLEYFPSQMLRTGNNFTFSYTFEDVPFHSSYAHSQSLDRLMNPLIDQYLYFLSRTNTPSGTTTQSRLQFSQAGASDIRDQSRNWLPGPCYRQQRVSKTSADNNNSEFSWTGATKYHLNGRDSLVNPGPAMASHKDDEEKFFPQSGVLIFGKQGSEKTNVDIEKVMITDEEEIRTTNPVATEQYGSVSTNLQRGNAAADTRPHDQAARQAATADVNTQGVLPGMVWQDRDVYLQGPIWAKIPHTDGHFHPSPLMGGFGLKHPPPQILIKNTPVPANPSTTFSAAKFASFITQYSTGQVSVEIEWELQKENSKRWNPEIQFTSNYNKSVNVDFTVDTNGVYSEPRPIGTRFLTRNL

SEQ ID NO: 4 - protein, 747 aa, Artificial Sequence
  AAV2 capsid protein VP1 with insertion
MAADGYLPDWLEDTLSEGIRQWWKLKPGPPPPKPAERHKDDSRGLVLPGYKYLGPFNGLDKGEPVNEADAAALEHDKAYDRQLDSGDNPYLKYNHADAEFQERLKEDTSFGGNLGRAVFQAKKRVLEPLGLVEEPVKTAPGKKRPVEHSPVEPDSSSGTGKAGQQPARKRLNFGQTGDADSVPDPQPLGQPPAAPSGLGTNTMATGSGAPMADNNEGADGVGNSSGNWHCDSTWMGDRVITTSTRTWALPTFNNHLYKQISSQSGASNDNHFFGYSTPWGYFDFNRFHCHFSPRDWQRLINNNWGFRPKRLNFKLFNIQVKEVTQNDGTTTIANNLTSTVQVFTDSEYQLPYVLGSAHQGCLPPFPADVFMVPQYGYLTLNNGSQAVGRSSFYCLEYFPSQMLRTGNNFTFSYTFEDVPFHSSYAHSQSLDRLMNPLIDQYLYFLSRTNTPSGTTTQSRLQFSQAGASDIRDQSRNWLPGPCYRQQRVSKTSADNNNSEFSWTGATKYHLNGRDSLVNPGPAMASHKDDEEKFFPQSGVLIFGKQGSEKTNVDIEKVMITDEEEIRTTNPVATEQYGSVSTNLQRGNAAAEHYNSTCAARQAATADVNTQGVLPGMVWQDRDVYLQGPIWAKIPHTDGHFHPSPLMGGFGLKHPPPQILIKNTPVPANPSTTFSAAKFASFITQYSTGQVSVEIEWELQKENSKRWNPEIQFTSNYNKSVNVDFTVDTNGVYSEPRPIGTRFLTRNL

SEQ ID NO: 5 - protein, 747 aa, Artificial Sequence
  AAV2 capsid protein VP1 with insertion
MAADGYLPDWLEDTLSEGIRQWWKLKPGPPPPKPAERHKDDSRGLVLPGYKYLGPFNGLDKGEPVNEADAAALEHDKAYDRQLDSGDNPYLKYNHADAEFQERLKEDTSFGGNLGRAVFQAKKRVLEPLGLVEEPVKTAPGKKRPVEHSPVEPDSSSGTGKAGQQPARKRLNFGQTGDADSVPDPQPLGQPPAAPSGLGTNTMATGSGAPMADNNEGADGVGNSSGNWHCDSTWMGDRVITTSTRTWALPTFNNHLYKQISSQSGASNDNHFFGYSTPWGYFDFNRFHCHFSPRDWQRLINNNWGFRPKRLNFKLFNIQVKEVTQNDGTTTIANNLTSTVQVFTDSEYQLPYVLGSAHQGCLPPFPADVFMVPQYGYLTLNNGSQAVGRSSFYCLEYFPSQMLRTGNNFTFSYTFEDVPFHSSYAHSQSLDRLMNPLIDQYLYFLSRTNTPSGTTTQSRLQFSQAGASDIRDQSRNWLPGPCYRQQRVSKTSADNNNSEFSWTGATKYHLNGRDSLVNPGPAMASHKDDEEKFFPQSGVLIFGKQGSEKTNVDIEKVMITDEEEIRTTNPVATEQYGSVSTNLQRGNAAAPNPNCTLAARQAATADVNTQGVLPGMVWQDRDVYLQGPIWAKIPHTDGHFHPSPLMGGFGLKHPPPQILIKNTPVPANPSTTFSAAKFASFITQYSTGQVSVEIEWELQKENSKRWNPEIQFTSNYNKSVNVDFTVDTNGVYSEPRPIGTRFLTRNL

SEQ ID NO: 6 - protein, 747 aa, Artificial Sequence
  AAV2 capsid protein VP1 with insertion
MAADGYLPDWLEDTLSEGIRQWWKLKPGPPPPKPAERHKDDSRGLVLPGYKYLGPFNGLDKGEPVNEADAAALEHDKAYDRQLDSGDNPYLKYNHADAEFQERLKEDTSFGGNLGRAVFQAKKRVLEPLGLVEEPVKTAPGKKRPVEHSPVEPDSSSGTGKAGQQPARKRLNFGQTGDADSVPDPQPLGQPPAAPSGLGTNTMATGSGAPMADNNEGADGVGNSSGNWHCDSTWMGDRVITTSTRTWALPTFNNHLYKQISSQSGASNDNHFFGYSTPWGYFDFNRFHCHFSPRDWQRLINNNWGFRPKRLNFKLFNIQVKEVTQNDGTTTIANNLTSTVQVFTDSEYQLPYVLGSAHQGCLPPFPADVFMVPQYGYLTLNNGSQAVGRSSFYCLEYFPSQMLRTGNNFTFSYTFEDVPFHSSYAHSQSLDRLMNPLIDQYLYFLSRTNTPSGTTTQSRLQFSQAGASDIRDQSRNWLPGPCYRQQRVSKTSADNNNSEFSWTGATKYHLNGRDSLVNPGPAMASHKDDEEKFFPQSGVLIFGKQGSEKTNVDIEKVMITDEEEIRTTNPVATEQYGSVSTNLQRGNAAATPPSITAAARQAATADVNTQGVLPGMVWQDRDVYLQGPIWAKIPHTDGHFHPSPLMGGFGLKHPPPQILIKNTPVPANPSTTFSAAKFASFITQYSTGQVSVEIEWELQKENSKRWNPEIQFTSNYNKSVNVDFTVDTNGVYSEPRPIGTRFLTRNL

SEQ ID NO: 7 - protein, 747 aa, Artificial Sequence
  AAV2 capsid protein VP1 with insertion
MAADGYLPDWLEDTLSEGIRQWWKLKPGPPPPKPAERHKDDSRGLVLPGYKYLGPFNGLDKGEPVNEADAAALEHDKAYDRQLDSGDNPYLKYNHADAEFQERLKEDTSFGGNLGRAVFQAKKRVLEPLGLVEEPVKTAPGKKRPVEHSPVEPDSSSGTGKAGQQPARKRLNFGQTGDADSVPDPQPLGQPPAAPSGLGTNTMATGSGAPMADNNEGADGVGNSSGNWHCDSTWMGDRVITTSTRTWALPTFNNHLYKQISSQSGASNDNHFFGYSTPWGYFDFNRFHCHFSPRDWQRLINNNWGFRPKRLNFKLFNIQVKEVTQNDGTTTIANNLTSTVQVFTDSEYQLPYVLGSAHQGCLPPFPADVFMVPQYGYLTLNNGSQAVGRSSFYCLEYFPSQMLRTGNNFTFSYTFEDVPFHSSYAHSQSLDRLMNPLIDQYLYFLSRTNTPSGTTTQSRLQFSQAGASDIRDQSRNWLPGPCYRQQRVSKTSADNNNSEFSWTGATKYHLNGRDSLVNPGPAMASHKDDEEKFFPQSGVLIFGKQGSEKTNVDIEKVMITDEEEIRTTNPVATEQYGSVSTNLQRGNAAACGESSYLAARQAATADVNTQGVLPGMVWQDRDVYLQGPIWAKIPHTDGHFHPSPLMGGFGLKHPPPQILIKNTPVPANPSTTFSAAKFASFITQYSTGQVSVEIEWELQKENSKRWNPEIQFTSNYNKSVNVDFTVDTNGVYSEPRPIGTRFLTRNL

SEQ ID NO: 8 - protein, 747 aa, Artificial Sequence
  AAV2 capsid protein VP1 with insertion
MAADGYLPDWLEDTLSEGIRQWWKLKPGPPPPKPAERHKDDSRGLVLPGYKYLGPFNGLDKGEPVNEADAAALEHDKAYDRQLDSGDNPYLKYNHADAEFQERLKEDTSFGGNLGRAVFQAKKRVLEPLGLVEEPVKTAPGKKRPVEHSPVEPDSSSGTGKAGQQPARKRLNFGQTGDADSVPDPQPLGQPPAAPSGLGTNTMATGSGAPMADNNEGADGVGNSSGNWHCDSTWMGDRVITTSTRTWALPTFNNHLYKQISSQSGASNDNHFFGYSTPWGYFDFNRFHCHFSPRDWQRLINNNWGFRPKRLNFKLFNIQVKEVTQNDGTTTIANNLTSTVQVFTDSEYQLPYVLGSAHQGCLPPFPADVFMVPQYGYLTLNNGSQAVGRSSFYCLEYFPSQMLRTGNNFTFSYTFEDVPFHSSYAHSQSLDRLMNPLIDQYLYFLSRTNTPSGTTTQSRLQFSQAGASDIRDQSRNWLPGPCYRQQRVSKTSADNNNSEFSWTGATKYHLNGRDSLVNPGPAMASHKDDEEKFFPQSGVLIFGKQGSEKTNVDIEKVMITDEEEIRTTNPVATEQYGSVSTNLQRGNAAAPRTPHTAAARQAATADVNTQGVLPGMVWQDRDVYLQGPIWAKIPHTDGHFHPSPLMGGFGLKHPPPQILIKNTPVPANPSTTFSAAKFASFITQYSTGQVSVEIEWELQKENSKRWNPEIQFTSNYNKSVNVDFTVDTNGVYSEPRPIGTRFLTRNL

SEQ ID NO: 9 - protein, 747 aa, Artificial Sequence
  AAV2 capsid protein VP1 with insertion
MAADGYLPDWLEDTLSEGIRQWWKLKPGPPPPKPAERHKDDSRGLVLPGYKYLGPFNGLDKGEPVNEADAAALEHDKAYDRQLDSGDNPYLKYNHADAEFQERLKEDTSFGGNLGRAVFQAKKRVLEPLGLVEEPVKTAPGKKRPVEHSPVEPDSSSGTGKAGQQPARKRLNFGQTGDADSVPDPQPLGQPPAAPSGLGTNTMATGSGAPMADNNEGADGVGNSSGNWHCDSTWMGDRVITTSTRTWALPTFNNHLYKQISSQSGASNDNHFFGYSTPWGYFDFNRFHCHFSPRDWQRLINNNWGFRPKRLNFKLFNIQVKEVTQNDGTTTIANNLTSTVQVFTDSEYQLPYVLGSAHQGCLPPFPADVFMVPQYGYLTLNNGSQAVGRSSFYCLEYFPSQMLRTGNNFTFSYTFEDVPFHSSYAHSQSLDRLMNPLIDQYLYFLSRTNTPSGTTTQSRLQFSQAGASDIRDQSRNWLPGPCYRQQRVSKTSADNNNSEFSWTGATKYHLNGRDSLVNPGPAMASHKDDEEKFFPQSGVLIFGKQGSEKTNVDIEKVMITDEEEIRTTNPVATEQYGSVSTNLQRGNAAAELCDGFAAARQAATADVNTQGVLPGMVWQDRDVYLQGPIWAKIPHTDGHFHPSPLMGGFGLKHPPPQILIKNTPVPANPSTTFSAAKFASFITQYSTGQVSVEIEWELQKENSKRWNPEIQFTSNYNKSVNVDFTVDTNGVYSEPRPIGTRFLTRNL

SEQ ID NO: 10 - protein, 7 aa, Artificial Sequence
  heptamer insert
SASEAST

SEQ ID NO: 11 - protein, 7 aa, Artificial Sequence
  heptamer insert
DTRPHDQ

SEQ ID NO: 12 - protein, 7 aa, Artificial Sequence
  heptamer insert
EHYNSTC

SEQ ID NO: 13 - protein, 7 aa, Artificial Sequence
  heptamer insert
PNPNCTL

SEQ ID NO: 14 - protein, 7 aa, Artificial Sequence
  heptamer insert
TPPSITA

SEQ ID NO: 15 - protein, 7 aa, Artificial Sequence
  heptamer insert
CGESSYL

SEQ ID NO: 16 - protein, 7 aa, Artificial Sequence
  heptamer insert
PRTPHTA

SEQ ID NO: 17 - protein, 7 aa, Artificial Sequence
  heptamer insert
ELCDGFA

SEQ ID NO: 18 - protein, 7 aa, Artificial Sequence
  heptamer insert
HHNDRAP

SEQ ID NO: 19 - protein, 7 aa, Artificial Sequence
  heptamer insert
DGNLHKS

SEQ ID NO: 20 - protein, 7 aa, Artificial Sequence
  heptamer insert
HSDSSKP

SEQ ID NO: 21 - protein, 7 aa, Artificial Sequence
  heptamer insert
TLTGLCP

SEQ ID NO: 22 - protein, 7 aa, Artificial Sequence
  heptamer insert
NHAPNHC

SEQ ID NO: 23 - protein, 7 aa, Artificial Sequence
  heptamer insert
DRRPGIC

SEQ ID NO: 24 - protein, 7 aa, Artificial Sequence
  heptamer insert
VDATCMQ

SEQ ID NO: 25 - DNA, 54 bp, Artificial Sequence
  single-stranded randomized 7mer pool with NNB codons
  misc_feature (14)..(15): n is a, c, g, or t
  misc_feature (17)..(18): n is a, c, g, or t
  misc_feature (20)..(21): n is a, c, g, or t
  misc_feature (23)..(24): n is a, c, g, or t
  misc_feature (26)..(27): n is a, c, g, or t
  misc_feature (29)..(30): n is a, c, g, or t
  misc_feature (32)..(33): n is a, c, g, or t
ttggcgcgccgcvnnvnnvnnvnnvnnvnnvnnggcggccgcttttttccttga

SEQ ID NO: 26 - DNA, 15 bp, Artificial Sequence
  antisense primer
ctcaaggaaaaaagc

SEQ ID NO: 27 - DNA, 2208 bp, adeno-associated virus 2
atggctgccgatggttatcttccagattggctcgaggacactctctctgaaggaataagacagtggtggaagctcaaacctggcccaccaccaccaaagcccgcagagcggcataaggacgacagcaggggtcttgtgcttcctgggtacaagtacctcggacccttcaacggactcgacaagggagagccggtcaacgaggcagacgccgcggccctcgagcacgacaaagcctacgaccggcagctcgacagcggagacaacccgtacctcaagtacaaccacgccgacgcggagtttcaggagcgccttaaagaagatacgtcttttgggggcaacctcggacgagcagtcttccaggcgaaaaagagggttcttgaacctctgggcctggttgaggaacctgttaagacggctccgggaaaaaagaggccggtagagcactctcctgtggagccagactcctcctcgggaaccggaaaggcgggccagcagcctgcaagaaaaagattgaattttggtcagactggagacgcagactcagtacctgacccccagcctctcggacagccaccagcagccccctctggtctgggaactaatacgatggctacaggcagtggcgcaccaatggcagacaataacgagggcgccgacggagtgggtaattcctccggaaattggcattgcgattccacatggatgggcgacagagtcatcaccaccagcacccgaacctgggccctgcccaccttcaacaaccacctgtacaaacaaatttccagccaatcaggagcttcgaacgacaatcacttctttggctacagcaccccttgggggtattttgacttcaacagattccactgccacttttcaccacgtgactggcaaagactcatcaacaacaactggggattccgacccaagagactcaacttcaagctctttaacattcaagtcaaagaggtcacgcagaatgacggtacgacgacgattgccaataaccttaccagcacggttcaggtgtttactgactcggagtaccagctcccgtacgtcctcggctcggcgcatcaaggatgcctcccgccgttcccagcagacgtcttcatggtgccacagtatggatacctcaccctgaacaacgggagtcaggcagtaggacgctcttcattttactgcctggagtactttccttctcagatgctgcgtaccggaaacaactttaccttcagctacacttttgaggacgttcctttccacagcagctacgctcacagccagagtctggaccgtctcatgaatcctctcatcgaccagtacctgtatttcttaagcagaacaaacactccaagtggaaccaccacgcagtcaaggcttcagttttctcaggccggagcgagtgacattcgggaccagtctaggaactggcttcctggaccctgttaccgccagcagcgagtatcaaagacatctgcggataacaacaacagtgaattctcgtggaccggtgctaccaagtaccacctcaatggcagagactctctggtgaatccgggcccggccatggcaagccacaaggacgatgaagaaaagttttttcctcagagcggggttctcatctttgggaagcaaggctcagagaaaacaaatgtggacattgaaaaggtcatgattacagacgaagaggaaatcaggacaaccaatcccgtggctacggagcagtatggttctgtatctaccaacctccagagaggcaacagacaagcagctaccgcagatgtcaacacacaaggcgttcttccaggcatggtctggcaggacagagatgtgtaccttcaggggcccatctgggcaaagattccacacacggacggacattttcacccctctcccctcatgggtggattcggacttaaacaccctcctccacagattctcatcaagaacaccccggtacctgcgaatccttcgaccaccttcagtgcggcaaagtttgcttccttcatcacacagtactccacgggacaggtcagcgtggagatcgagtgggagctgcagaaggaaaacagcaaacgctggaatcccgaaattcagttcacttcgaactacaacaagtctgttaatgtggactttactgtggacactaatggcgtgtattcagagcctcgccccattggtaccagattcctgactcgtaatctgtaa

SEQ ID NO: 28 - protein, 12 aa, Artificial Sequence
  alanin spacer
AAASASEASTAA